European Patent Specification EP 3 875 109 B1, published October 2, 2024. Title: application of anti-platelet thrombolysin in preparing drug for treating anemia. Applicant: ZHAOKE PHARMACEUTICAL (HEFEI) COMPANY LIMTED. The sequence listing filed with the application follows.

SEQUENCE LISTING (2 sequences)

SEQ ID NO: 1 - protein, 130 aa, artificial sequenc
DVDCLPGWSAYDQSCYRVFKLLKTWDDAEKFCTERPKGGHLVSIESAGERDFVAQLVSENKQTDNVWLGLKIQSKGQQCSTEWTDGSSVSYENFSEYQSKKCFVEKNTGFRTWLNLNCGSEYAFVCKSPP

SEQ ID NO: 2 - protein, 125 aa, artificial sequenc
GFCCPLRWSSYEGHCYLVVKEKKTWDDAEKFCTEQRKGGHLVSVHSREEADFLVHLAYPILDLSLIWMGLSNMWNDCKREWSDGTKLDFKAWAKTSDCLIGKTDDNQWLNMDCSKKHYFVCKFKL